European Patent Application EP 4 471 065 A1, published December 4, 2024. Title: GPRC5D ANTIBODY AND USE THEREOF. Applicant: CARSGEN LIFE SCIENCES CO., LTD. The sequence listing filed with the application follows.

SEQUENCE LISTING (91 sequences)

SEQ ID NO: 1 - protein, 5 aa, synthetic construct
SYAMS

SEQ ID NO: 2 - protein, 17 aa, synthetic construct
AISGSGGSTYYADSVKG

SEQ ID NO: 3 - protein, 10 aa, synthetic construct
GWPSPVTFDY

SEQ ID NO: 4 - protein, 12 aa, synthetic construct
RASQSVSSSYLA

SEQ ID NO: 5 - protein, 7 aa, synthetic construct
GASSRAT

SEQ ID NO: 6 - protein, 9 aa, synthetic construct
QQYKSHPIT

SEQ ID NO: 7 - protein, 11 aa, synthetic construct
GVRWVPLAFDY

SEQ ID NO: 8 - protein, 9 aa, synthetic construct
QQYGRSPMT

SEQ ID NO: 9 - protein, 10 aa, synthetic construct
GYPVPVSFDY

SEQ ID NO: 10 - protein, 9 aa, synthetic construct
QQYGNRPIT

SEQ ID NO: 11 - protein, 5 aa, synthetic construct
GYTMN

SEQ ID NO: 12 - protein, 17 aa, synthetic construct
LINPYNGGTSYNQKFKG

SEQ ID NO: 13 - protein, 9 aa, synthetic construct
GGFRAWFAF

SEQ ID NO: 14 - protein, 11 aa, synthetic construct
RASQDIGSNLN

SEQ ID NO: 15 - protein, 7 aa, synthetic construct
ATSILDS

SEQ ID NO: 16 - protein, 9 aa, synthetic construct
LQYATFPNT

SEQ ID NO: 17 - protein, 5 aa, synthetic construct
NYGMS

SEQ ID NO: 18 - protein, 17 aa, synthetic construct
TINSNGGNTYYPDSVKG

SEQ ID NO: 19 - protein, 8 aa, synthetic construct
AYSLTMDY

SEQ ID NO: 20 - protein, 16 aa, synthetic construct
RSSQSLVHSNGNTYLH

SEQ ID NO: 21 - protein, 7 aa, synthetic construct
KVSNRFS

SEQ ID NO: 22 - protein, 9 aa, synthetic construct
SQSTHVPPT

SEQ ID NO: 23 - protein, 119 aa, synthetic construct
EVQLLESGGGLVQPGGSLRLSCAASGFTFSSYAMSWVRQAPGKGLEWVSAISGSGGSTYYADSVKGRFTISRDNSKNTLYLQMNSLRAEDTAVYYCARGWPSPVTFDYWGQGTLVTVSS

SEQ ID NO: 24 - DNA, 357 bp, synthetic construct
  source 1..357: mol_type = other DNA
gaggtgcaattgctggagtctgggggaggcttggtacagcctggggggtccctgagactctcctgtgcagcctccggattcacctttagcagttatgccatgagctgggtccgccaggctccagggaaggggctggagtgggtctcagctattagtggtagtggtggtagcacatactacgcagactccgtgaagggccggttcaccatctccagagacaattccaagaacacgctgtatctgcagatgaacagcctgagagccgaggacacggccgtatattactgtgcgcgtggttggccatctccagttactttcgactactggggccaaggaaccctggtcaccgtctcgagt

SEQ ID NO: 25 - protein, 109 aa, synthetic construct
EIVLTQSPGTLSLSPGERATLSCRASQSVSSSYLAWYQQKPGQAPRLLIYGASSRATGIPDRFSGSGSGTDFTLTISRLEPEDFAVYYCQQYKSHPITFGQGTKVEIKR

SEQ ID NO: 26 - DNA, 327 bp, synthetic construct
  source 1..327: mol_type = other DNA
gaaatcgtgttaacgcagtctccaggcaccctgtctttgtctccaggggaaagagccaccctctcttgcagggccagtcagagtgttagcagcagctacttagcctggtaccagcagaaacctggccaggctcccaggctcctcatctatggagcatccagcagggccactggcatcccagacaggttcagtggcagtggatccgggacagacttcactctcaccatcagcagactggagcctgaagattttgcagtgtattactgtcagcagtacaaatctcatccaatcacgttcggccaggggaccaaagtggaaatcaaacgt

SEQ ID NO: 27 - protein, 120 aa, synthetic construct
EVQLLESGGGLVQPGGSLRLSCAASGFTFSSYAMSWVRQAPGKGLEWVSAISGSGGSTYYADSVKGRFTISRDNSKNTLYLQMNSLRAEDTAVYYCAKGVRWVPLAFDYWGQGTLVTVSS

SEQ ID NO: 28 - DNA, 360 bp, synthetic construct
  source 1..360: mol_type = other DNA
gaggtgcaattgctggagtctgggggaggcttggtacagcctggggggtccctgagactctcctgtgcagcctccggattcacctttagcagttatgccatgagctgggtccgccaggctccagggaaggggctggagtgggtctcagctattagtggtagtggtggtagcacatactacgcagactccgtgaagggccggttcaccatctccagagacaattccaagaacacgctgtatctgcagatgaacagcctgagagccgaggacacggccgtatattactgtgcgaaaggtgttcgttgggttccactggcattcgactactggggccaaggaaccctggtcaccgtctcgagt

SEQ ID NO: 29 - protein, 109 aa, synthetic construct
EIVLTQSPGTLSLSPGERATLSCRASQSVSSSYLAWYQQKPGQAPRLLIYGASSRATGIPDRFSGSGSGTDFTLTISRLEPEDFAVYYCQQYGRSPMTFGQGTKVEIKR

SEQ ID NO: 30 - DNA, 327 bp, synthetic construct
  source 1..327: mol_type = other DNA
gaaatcgtgttaacgcagtctccaggcaccctgtctttgtctccaggggaaagagccaccctctcttgcagggccagtcagagtgttagcagcagctacttagcctggtaccagcagaaacctggccaggctcccaggctcctcatctatggagcatccagcagggccactggcatcccagacaggttcagtggcagtggatccgggacagacttcactctcaccatcagcagactggagcctgaagattttgcagtgtattactgtcagcagtacggtagatctccaatgacgttcggccaggggaccaaagtggaaatcaaacgt

SEQ ID NO: 31 - protein, 119 aa, synthetic construct
EVQLLESGGGLVQPGGSLRLSCAASGFTFSSYAMSWVRQAPGKGLEWVSAISGSGGSTYYADSVKGRFTISRDNSKNTLYLQMNSLRAEDTAVYYCARGYPVPVSFDYWGQGTLVTVSS

SEQ ID NO: 32 - DNA, 357 bp, synthetic construct
  source 1..357: mol_type = other DNA
gaggtgcaattgctggagtctgggggaggcttggtacagcctggggggtccctgagactctcctgtgcagcctccggattcacctttagcagttatgccatgagctgggtccgccaggctccagggaaggggctggagtgggtctcagctattagtggtagtggtggtagcacatactacgcagactccgtgaagggccggttcaccatctccagagacaattccaagaacacgctgtatctgcagatgaacagcctgagagccgaggacacggccgtatattactgtgcgcgtggttacccagttccagtttctttcgactactggggccaaggaaccctggtcaccgtctcgagt

SEQ ID NO: 33 - protein, 109 aa, synthetic construct
EIVLTQSPGTLSLSPGERATLSCRASQSVSSSYLAWYQQKPGQAPRLLIYGASSRATGIPDRFSGSGSGTDFTLTISRLEPEDFAVYYCQQYGNRPITFGQGTKVEIKR

SEQ ID NO: 34 - DNA, 327 bp, synthetic construct
  source 1..327: mol_type = other DNA
gaaatcgtgttaacgcagtctccaggcaccctgtctttgtctccaggggaaagagccaccctctcttgcagggccagtcagagtgttagcagcagctacttagcctggtaccagcagaaacctggccaggctcccaggctcctcatctatggagcatccagcagggccactggcatcccagacaggttcagtggcagtggatccgggacagacttcactctcaccatcagcagactggagcctgaagattttgcagtgtattactgtcagcagtacggtaacagaccaatcacgttcggccaggggaccaaagtggaaatcaaacgt

SEQ ID NO: 35 - protein, 118 aa, synthetic construct
EVQLQQSGPEVVKPGASMKISCKASGYSFTGYTMNWVKQSHGKNFEWIGLINPYNGGTSYNQKFKGKATLTVDKSSSTAYMELLSLTSEDSAVYYCTRGGFRAWFAFWGQGTLVTVSA

SEQ ID NO: 36 - DNA, 354 bp, synthetic construct
  source 1..354: mol_type = other DNA
gaggtccagctgcaacagtctggacctgaggtggtgaagcctggagcttcaatgaagatatcctgcaaggcttctggttactcattcactggctacaccatgaactgggtgaagcagagccatggaaagaattttgagtggattggacttattaatccttacaatggtggtactagttacaaccagaaattcaagggcaaggccacattaactgtggacaagtcatccagcacagcctacatggaactcctcagtctgacatctgaggactctgcagtctattattgtacaagaggaggatttcgagcctggtttgctttctggggccaggggactctggtcactgtctctgca

SEQ ID NO: 37 - protein, 108 aa, synthetic construct
DIQMTQSPSSLSASLGERVSLTCRASQDIGSNLNWLQQEPDGTIKRLIYATSILDSGVPKRFSGSRSGSDYSLTISSLESEDFVDYYCLQYATFPNTFGGGTKLEIKR

SEQ ID NO: 38 - DNA, 324 bp, synthetic construct
  source 1..324: mol_type = other DNA
gacatccagatgacccagtctccatcctccttatctgcctctctgggagaaagagtcagtctcacttgtcgggcaagtcaggacattggtagtaacttaaactggcttcagcaggaaccagatggaactattaaacgcctgatctacgccacatccattttagattctggtgtccccaaaaggttcagtggcagtaggtctgggtcagattattctctcaccatcagcagccttgagtctgaagattttgtagactattactgtctacaatatgctacttttccgaacacgttcggaggggggaccaagctggaaataaaacgg

SEQ ID NO: 39 - protein, 117 aa, synthetic construct
VVKLVESGGGLVQPGGSLKLSCAASGFTFSNYGMSWVRQTPDTRLELVATINSNGGNTYYPDSVKGRFTISRDNAKNTLYLQMSSLKSEDTAIYYCVRAYSLTMDYWGQGTSVTVSS

SEQ ID NO: 40 - DNA, 351 bp, synthetic construct
  source 1..351: mol_type = other DNA
gtggtgaagctggtggagtcggggggaggcttagtgcagcctggagggtccctgaaactctcctgtgcagcctctggattcactttcagtaactatggcatgtcttgggttcgccagactccagacacgaggctggagttggtcgcaaccattaatagtaatggtggtaacacctattatccagacagtgtgaagggccgattcaccatctccagagacaatgccaagaacaccctgtacctgcaaatgagcagtctgaagtctgaggacacagccatatattactgtgttagagcttactccctgactatggactactggggtcaaggaacctcagtcaccgtctcctca

SEQ ID NO: 41 - protein, 113 aa, synthetic construct
DVVMTQTPLSLPVSLGDQASISCRSSQSLVHSNGNTYLHWYLQKPGQSPKLLIYKVSNRFSGVPDRFSGSGSGTDFTLKIIRVEAEDLGVYFCSQSTHVPPTFRAGTKLELKR

SEQ ID NO: 42 - DNA, 339 bp, synthetic construct
  source 1..339: mol_type = other DNA
gatgttgtgatgacccaaactccactctccctgcctgtcagtcttggagatcaagcctccatctcttgtagatctagtcagagccttgtacacagtaatggaaacacctatttacattggtacctgcagaagccaggccagtctccaaagctcctgatctacaaagtttccaaccgattttctggggtcccagacaggttcagtggcagtggatcagggacagatttcacactcaagatcatcagagtggaggctgaggatctgggagtttatttctgctctcaaagtacacatgttcctcctacgttccgtgctgggaccaagctggagctgaaacgg

SEQ ID NO: 43 - protein, 243 aa, synthetic construct
EVQLLESGGGLVQPGGSLRLSCAASGFTFSSYAMSWVRQAPGKGLEWVSAISGSGGSTYYADSVKGRFTISRDNSKNTLYLQMNSLRAEDTAVYYCARGWPSPVTFDYWGQGTLVTVSSGGGGSGGGGSGGGGSEIVLTQSPGTLSLSPGERATLSCRASQSVSSSYLAWYQQKPGQAPRLLIYGASSRATGIPDRFSGSGSGTDFTLTISRLEPEDFAVYYCQQYKSHPITFGQGTKVEIKR

SEQ ID NO: 44 - DNA, 729 bp, synthetic construct
  source 1..729: mol_type = other DNA
gaggtgcaattgctggagtctgggggaggcttggtacagcctggggggtccctgagactctcctgtgcagcctccggattcacctttagcagttatgccatgagctgggtccgccaggctccagggaaggggctggagtgggtctcagctattagtggtagtggtggtagcacatactacgcagactccgtgaagggccggttcaccatctccagagacaattccaagaacacgctgtatctgcagatgaacagcctgagagccgaggacacggccgtatattactgtgcgcgtggttggccatctccagttactttcgactactggggccaaggaaccctggtcaccgtctcgagtggtggaggcggttcaggcggaggtggttctggcggtggcggatcggaaatcgtgttaacgcagtctccaggcaccctgtctttgtctccaggggaaagagccaccctctcttgcagggccagtcagagtgttagcagcagctacttagcctggtaccagcagaaacctggccaggctcccaggctcctcatctatggagcatccagcagggccactggcatcccagacaggttcagtggcagtggatccgggacagacttcactctcaccatcagcagactggagcctgaagattttgcagtgtattactgtcagcagtacaaatctcatccaatcacgttcggccaggggaccaaagtggaaatcaaacgt

SEQ ID NO: 45 - protein, 223 aa, synthetic construct
EVQLLESGGGLVQPGGSLRLSCAASGFTFSSYAMSWVRQAPGKGLEWVSAISGSGGSTYYADSVKGRFTISRDNSKNTLYLQMNSLRAEDTAVYYCARGWPSPVTFDYWGQGTLVTVSSASTKGPSVFPLAPSSKSTSGGTAALGCLVKDYFPEPVTVSWNSGALTSGVHTFPAVLQSSGLYSLSSVVTVPSSSLGTQTYICNVNHKPSNTKVDKKVEPKSCD

SEQ ID NO: 46 - DNA, 669 bp, synthetic construct
  source 1..669: mol_type = other DNA
gaggtgcaattgctggagtctgggggaggcttggtacagcctggggggtccctgagactctcctgtgcagcctccggattcacctttagcagttatgccatgagctgggtccgccaggctccagggaaggggctggagtgggtctcagctattagtggtagtggtggtagcacatactacgcagactccgtgaagggccggttcaccatctccagagacaattccaagaacacgctgtatctgcagatgaacagcctgagagccgaggacacggccgtatattactgtgcgcgtggttggccatctccagttactttcgactactggggccaaggaaccctggtcaccgtctcgagtgctagcaccaaaggcccatcggtcttccccctggcaccctcctccaagagcacctctgggggcacagcggccctgggctgcctggtcaaggactacttccccgaaccggtgacggtgtcgtggaactcaggcgccctgaccagcggcgtgcacaccttcccggctgtcctacagtcctcaggactctactccctcagcagcgtggtgaccgtgccctccagcagcttgggcacccagacctacatctgcaacgtgaatcacaagcccagcaacaccaaagtggacaagaaagttgagcccaaatcttgtgac

SEQ ID NO: 47 - protein, 215 aa, synthetic construct
EIVLTQSPGTLSLSPGERATLSCRASQSVSSSYLAWYQQKPGQAPRLLIYGASSRATGIPDRFSGSGSGTDFTLTISRLEPEDFAVYYCQQYKSHPITFGQGTKVEIKRTVAAPSVFIFPPSDEQLKSGTASVVCLLNNFYPREAKVQWKVDNALQSGNSQESVTEQDSKDSTYSLSSTLTLSKADYEKHKVYACEVTHQGLSSPVTKSFNRGEC

SEQ ID NO: 48 - DNA, 645 bp, synthetic construct
  source 1..645: mol_type = other DNA
gaaatcgtgttaacgcagtctccaggcaccctgtctttgtctccaggggaaagagccaccctctcttgcagggccagtcagagtgttagcagcagctacttagcctggtaccagcagaaacctggccaggctcccaggctcctcatctatggagcatccagcagggccactggcatcccagacaggttcagtggcagtggatccgggacagacttcactctcaccatcagcagactggagcctgaagattttgcagtgtattactgtcagcagtacaaatctcatccaatcacgttcggccaggggaccaaagtggaaatcaaacgtacggtggctgcaccatctgtcttcatcttcccgccatctgatgagcagttgaaatctggaactgcctctgttgtgtgcctgctgaataacttctatcccagagaggccaaagtacagtggaaggtggataacgccctccaatcgggtaactcccaggagagtgtcacagagcaggacagcaaggacagcacctacagcctcagcagcaccctgacgctgagcaaagcagactacgagaaacacaaagtctacgcctgcgaagtcacccatcagggcctgagctcgcccgtcacaaagagcttcaacaggggagagtgt

SEQ ID NO: 49 - protein, 224 aa, synthetic construct
EVQLLESGGGLVQPGGSLRLSCAASGFTFSSYAMSWVRQAPGKGLEWVSAISGSGGSTYYADSVKGRFTISRDNSKNTLYLQMNSLRAEDTAVYYCAKGVRWVPLAFDYWGQGTLVTVSSASTKGPSVFPLAPSSKSTSGGTAALGCLVKDYFPEPVTVSWNSGALTSGVHTFPAVLQSSGLYSLSSVVTVPSSSLGTQTYICNVNHKPSNTKVDKKVEPKSCD

SEQ ID NO: 50 - DNA, 672 bp, synthetic construct
  source 1..672: mol_type = other DNA
gaggtgcaattgctggagtctgggggaggcttggtacagcctggggggtccctgagactctcctgtgcagcctccggattcacctttagcagttatgccatgagctgggtccgccaggctccagggaaggggctggagtgggtctcagctattagtggtagtggtggtagcacatactacgcagactccgtgaagggccggttcaccatctccagagacaattccaagaacacgctgtatctgcagatgaacagcctgagagccgaggacacggccgtatattactgtgcgaaaggtgttcgttgggttccactggcattcgactactggggccaaggaaccctggtcaccgtctcgagtgctagcaccaaaggcccatcggtcttccccctggcaccctcctccaagagcacctctgggggcacagcggccctgggctgcctggtcaaggactacttccccgaaccggtgacggtgtcgtggaactcaggcgccctgaccagcggcgtgcacaccttcccggctgtcctacagtcctcaggactctactccctcagcagcgtggtgaccgtgccctccagcagcttgggcacccagacctacatctgcaacgtgaatcacaagcccagcaacaccaaagtggacaagaaagttgagcccaaatcttgtgac

SEQ ID NO: 51 - protein, 215 aa, synthetic construct
EIVLTQSPGTLSLSPGERATLSCRASQSVSSSYLAWYQQKPGQAPRLLIYGASSRATGIPDRFSGSGSGTDFTLTISRLEPEDFAVYYCQQYGRSPMTFGQGTKVEIKRTVAAPSVFIFPPSDEQLKSGTASVVCLLNNFYPREAKVQWKVDNALQSGNSQESVTEQDSKDSTYSLSSTLTLSKADYEKHKVYACEVTHQGLSSPVTKSFNRGEC

SEQ ID NO: 52 - DNA, 645 bp, synthetic construct
  source 1..645: mol_type = other DNA
gaaatcgtgttaacgcagtctccaggcaccctgtctttgtctccaggggaaagagccaccctctcttgcagggccagtcagagtgttagcagcagctacttagcctggtaccagcagaaacctggccaggctcccaggctcctcatctatggagcatccagcagggccactggcatcccagacaggttcagtggcagtggatccgggacagacttcactctcaccatcagcagactggagcctgaagattttgcagtgtattactgtcagcagtacggtagatctccaatgacgttcggccaggggaccaaagtggaaatcaaacgtacggtggctgcaccatctgtcttcatcttcccgccatctgatgagcagttgaaatctggaactgcctctgttgtgtgcctgctgaataacttctatcccagagaggccaaagtacagtggaaggtggataacgccctccaatcgggtaactcccaggagagtgtcacagagcaggacagcaaggacagcacctacagcctcagcagcaccctgacgctgagcaaagcagactacgagaaacacaaagtctacgcctgcgaagtcacccatcagggcctgagctcgcccgtcacaaagagcttcaacaggggagagtgt

SEQ ID NO: 53 - protein, 223 aa, synthetic construct
EVQLLESGGGLVQPGGSLRLSCAASGFTFSSYAMSWVRQAPGKGLEWVSAISGSGGSTYYADSVKGRFTISRDNSKNTLYLQMNSLRAEDTAVYYCARGYPVPVSFDYWGQGTLVTVSSASTKGPSVFPLAPSSKSTSGGTAALGCLVKDYFPEPVTVSWNSGALTSGVHTFPAVLQSSGLYSLSSVVTVPSSSLGTQTYICNVNHKPSNTKVDKKVEPKSCD

SEQ ID NO: 54 - DNA, 669 bp, synthetic construct
  source 1..669: mol_type = other DNA
gaggtgcaattgctggagtctgggggaggcttggtacagcctggggggtccctgagactctcctgtgcagcctccggattcacctttagcagttatgccatgagctgggtccgccaggctccagggaaggggctggagtgggtctcagctattagtggtagtggtggtagcacatactacgcagactccgtgaagggccggttcaccatctccagagacaattccaagaacacgctgtatctgcagatgaacagcctgagagccgaggacacggccgtatattactgtgcgcgtggttacccagttccagtttctttcgactactggggccaaggaaccctggtcaccgtctcgagtgctagcaccaaaggcccatcggtcttccccctggcaccctcctccaagagcacctctgggggcacagcggccctgggctgcctggtcaaggactacttccccgaaccggtgacggtgtcgtggaactcaggcgccctgaccagcggcgtgcacaccttcccggctgtcctacagtcctcaggactctactccctcagcagcgtggtgaccgtgccctccagcagcttgggcacccagacctacatctgcaacgtgaatcacaagcccagcaacaccaaagtggacaagaaagttgagcccaaatcttgtgac

SEQ ID NO: 55 - protein, 215 aa, synthetic construct
EIVLTQSPGTLSLSPGERATLSCRASQSVSSSYLAWYQQKPGQAPRLLIYGASSRATGIPDRFSGSGSGTDFTLTISRLEPEDFAVYYCQQYGNRPITFGQGTKVEIKRTVAAPSVFIFPPSDEQLKSGTASVVCLLNNFYPREAKVQWKVDNALQSGNSQESVTEQDSKDSTYSLSSTLTLSKADYEKHKVYACEVTHQGLSSPVTKSFNRGEC

SEQ ID NO: 56 - DNA, 645 bp, synthetic construct
  source 1..645: mol_type = other DNA
gaaatcgtgttaacgcagtctccaggcaccctgtctttgtctccaggggaaagagccaccctctcttgcagggccagtcagagtgttagcagcagctacttagcctggtaccagcagaaacctggccaggctcccaggctcctcatctatggagcatccagcagggccactggcatcccagacaggttcagtggcagtggatccgggacagacttcactctcaccatcagcagactggagcctgaagattttgcagtgtattactgtcagcagtacggtaacagaccaatcacgttcggccaggggaccaaagtggaaatcaaacgtacggtggctgcaccatctgtcttcatcttcccgccatctgatgagcagttgaaatctggaactgcctctgttgtgtgcctgctgaataacttctatcccagagaggccaaagtacagtggaaggtggataacgccctccaatcgggtaactcccaggagagtgtcacagagcaggacagcaaggacagcacctacagcctcagcagcaccctgacgctgagcaaagcagactacgagaaacacaaagtctacgcctgcgaagtcacccatcagggcctgagctcgcccgtcacaaagagcttcaacaggggagagtgt

SEQ ID NO: 57 - protein, 244 aa, synthetic construct
EVQLVESGGGLIQPGGSLRLSCAASGFTFSNYAMNWVRQAPGKGLEWVSTINGRGSSTIYADSVKGRFTISRDNSKNTLYLQMNSLRAEDTATYYCARYISRGLGDSWGQGTLVTVSSGGGGSGGGGSGGGGSQSVVTQPPSMSAAPGQQVTISCSGGNSNIERNYVSWYLQLPGTAPKLVIFDNDRRPSGIPDRFSGSKSGTSATLGITGLQTGDEADYYCGTWDSSLRGWVFGGGTKLTVLG

SEQ ID NO: 58 - protein, 21 aa, synthetic construct
MALPVTALLLPLALLLHAARP

SEQ ID NO: 59 - protein, 45 aa, synthetic construct
TTTPAPRPPTPAPTIASQPLSLRPEACRPAAGGAVHTRGLDFACD

SEQ ID NO: 60 - protein, 24 aa, synthetic construct
IYIWAPLAGTCGVLLLSLVITLYC

SEQ ID NO: 61 - protein, 42 aa, synthetic construct
KRGRKKLLYIFKQPFMRPVQTTQEEDGCSCRFPEEEEGGCEL

SEQ ID NO: 62 - protein, 113 aa, synthetic construct
RVKFSRSADAPAYQQGQNQLYNELNLGRREEYDVLDKRRGRDPEMGGKPQRRKNPQEGLYNELQKDKMAEAYSEIGMKGERRRGKGHDGLYQGLSTATKDTYDALHMQALPPR

SEQ ID NO: 63 - protein, 467 aa, synthetic construct
EVQLLESGGGLVQPGGSLRLSCAASGFTFSSYAMSWVRQAPGKGLEWVSAISGSGGSTYYADSVKGRFTISRDNSKNTLYLQMNSLRAEDTAVYYCARGWPSPVTFDYWGQGTLVTVSSGGGGSGGGGSGGGGSEIVLTQSPGTLSLSPGERATLSCRASQSVSSSYLAWYQQKPGQAPRLLIYGASSRATGIPDRFSGSGSGTDFTLTISRLEPEDFAVYYCQQYKSHPITFGQGTKVEIKRTTTPAPRPPTPAPTIASQPLSLRPEACRPAAGGAVHTRGLDFACDIYIWAPLAGTCGVLLLSLVITLYCKRGRKKLLYIFKQPFMRPVQTTQEEDGCSCRFPEEEEGGCELRVKFSRSADAPAYQQGQNQLYNELNLGRREEYDVLDKRRGRDPEMGGKPQRRKNPQEGLYNELQKDKMAEAYSEIGMKGERRRGKGHDGLYQGLSTATKDTYDALHMQALPPR

SEQ ID NO: 64 - protein, 225 aa, synthetic construct
RDCGCKPCICTVPEVSSVFIFPPKPKDVLTITLTPKVTCVVVDISKDDPEVQFSWFVDDVEVHTAQTQPREEQFNSTFRSVSELPIMHQDWLNGKEFKCRVNSAAFPAPIEKTISKTKGRPKAPQVYTIPPPKEQMAKDKVSLTCMITDFFPEDITVEWQWNGQPAENYKNTQPIMDTDGSYFVYSKLNVQKSNWEAGNTFTCSVLHEGLHNHHTEKSLSHSPGK

SEQ ID NO: 65 - protein, 345 aa, synthetic construct
MYKDCIESTGDYFLLCDAEGPWGIILESLAILGIVVTILLLLAFLFLMRKIQDCSQWNVLPTQLLFLLSVLGLFGLAFAFIIELNQQTAPVRYFLFGVLFALCFSCLLAHASNLVKLVRGCVSFSWTTILCIAIGCSLLQIIIATEYVTLIMTRGMMFVNMTPCQLNVDFVVLLVYVLFLMALTFFVSKATFCGPCENWKQHGRLIFITVLFSIIIWVVWISMLLRGNPQFQRQPQWDDPVVCIALVTNAWVFLLLYIVPELCILYRSCRQECPLQGNACPVTAYQHSFQVENQELSRARDSDGAEEDVALTSYGTPIQPQTVDPTQECFIPQAKLSPQQDAGGV

SEQ ID NO: 66 - protein, 300 aa, synthetic construct
MYEDCVKSTEDYYLFCDNEGPWAIVLESLAVIGIVVTILLLLAFLFLMRKVQDCSQWNVLPTQFLFLLAVLGLFGLTFAFIIQLNHQTAPVRYFLFGVLFAICFSCLLAHASNLVKLVRGRVSFCWTTILFIAIGVSLLQTIIAIEYVTLIMTRGLMFEHMTPYQLNVDFVCLLIYVLFLMALTFFVSKATFCGPCENWKQHGRLIFATVLVSIIIWVVWISMLLRGNPQLQRQPHWDDAVICIGLVTNAWVFLLIYIIPELSILYRSCRQECPTQGNVCQVPVYQRSFRMDTQEPTREC

SEQ ID NO: 67 - DNA, 20 bp, synthetic construct
  source 1..20: mol_type = other DNA
acactgctggacagggatcc

SEQ ID NO: 68 - DNA, 25 bp, synthetic construct
  source 1..25: mol_type = other DNA
acagggctccatagttccattttac

SEQ ID NO: 69 - DNA, 22 bp, synthetic construct
  source 1..22: mol_type = other DNA
aggtgctgtctttgctgtcctg

SEQ ID NO: 70 - protein, 6 aa, synthetic construct
RRYAIS

SEQ ID NO: 71 - protein, 6 aa, synthetic construct
SRKALS

SEQ ID NO: 72 - protein, 17 aa, synthetic construct
AISGTGGSTKYADSVKG

SEQ ID NO: 73 - protein, 17 aa, synthetic construct
TINGRGGRTYYADSVKG

SEQ ID NO: 74 - protein, 12 aa, synthetic construct
RASQSVSRRYLA

SEQ ID NO: 75 - protein, 7 aa, synthetic construct
GGSRRAT

SEQ ID NO: 76 - protein, 119 aa, synthetic construct
EVQLLESGGGLVQPGGSLRLSCAASGFTFRRYAISWVRQAPGKGLEWVSAISGTGGSTKYADSVKGRFTISRDNSKNTLYLQMNSLRAEDTAVYYCARGWPSPVTFDYWGQGTLVTVSS

SEQ ID NO: 77 - DNA, 357 bp, synthetic construct
  source 1..357: mol_type = other DNA
gaggtgcaattgctggagtctgggggaggcttggtacagcctggggggtccctgagactctcctgtgcagcctccggattcacctttcgccgttatgcgatcagctgggtccgccaggctccagggaaggggctggagtgggtctcagctattagtggcactggaggtagcacaaagtacgcagactccgtgaagggccggttcaccatctccagagacaattccaagaacacgctgtatctgcagatgaacagcctgagagccgaggacacggccgtatattactgtgcgcgtggttggccatctccagttactttcgactactggggccaaggaaccctggtcaccgtctcgagt

SEQ ID NO: 78 - protein, 109 aa, synthetic construct
EIVLTQSPGTLSLSPGERATLSCRASQSVSRRYLAWYQQKPGQAPRLLIYGGSRRATGIPDRFSGSGSGTDFTLTISRLEPEDFAVYYCQQYKSHPITFGQGTKVEIKR

SEQ ID NO: 79 - DNA, 327 bp, synthetic construct
  source 1..327: mol_type = other DNA
gaaatcgtgttaacgcagtctccaggcaccctgtctttgtctccaggggaaagagccaccctctcttgcagggccagtcagagcgtcagtaggcgatacttagcctggtaccagcagaaacctggccaggctcccaggctcctcatctacggaggttcgcggagggccactggcatcccagacaggttcagtggcagtggatccgggacagacttcactctcaccatcagcagactggagcctgaagattttgcagtgtattactgtcagcagtacaaatctcatccaatcacgttcggccaggggaccaaagtggaaatcaaacgt

SEQ ID NO: 80 - protein, 119 aa, synthetic construct
EVQLLESGGGLVQPGGSLRLSCAASGFTFSRKALSWVRQAPGKGLEWVSTINGRGGRTYYADSVKGRFTISRDNSKNTLYLQMNSLRAEDTAVYYCARGWPSPVTFDYWGQGTLVTVSS

SEQ ID NO: 81 - DNA, 357 bp, synthetic construct
  source 1..357: mol_type = other DNA
gaggtgcaattgctggagtctgggggaggcttggtacagcctggggggtccctgagactctcctgtgcagcctccggattcacctttagcagaaaggccctaagctgggtccgccaggctccagggaaggggctggagtgggtctcaactattaatggtagaggtggtcgcacatactacgcagactccgtgaagggccggttcaccatctccagagacaattccaagaacacgctgtatctgcagatgaacagcctgagagccgaggacacggccgtatattactgtgcgcgtggttggccatctccagttactttcgactactggggccaaggaaccctggtcaccgtctcgagt

SEQ ID NO: 82 - protein, 243 aa, synthetic construct
EVQLLESGGGLVQPGGSLRLSCAASGFTFRRYAISWVRQAPGKGLEWVSAISGTGGSTKYADSVKGRFTISRDNSKNTLYLQMNSLRAEDTAVYYCARGWPSPVTFDYWGQGTLVTVSSGGGGSGGGGSGGGGSEIVLTQSPGTLSLSPGERATLSCRASQSVSSSYLAWYQQKPGQAPRLLIYGASSRATGIPDRFSGSGSGTDFTLTISRLEPEDFAVYYCQQYKSHPITFGQGTKVEIKR

SEQ ID NO: 83 - DNA, 729 bp, synthetic construct
  source 1..729: mol_type = other DNA
gaggtgcaattgctggagtctgggggaggcttggtacagcctggggggtccctgagactctcctgtgcagcctccggattcacctttcgccgttatgcgatcagctgggtccgccaggctccagggaaggggctggagtgggtctcagctattagtggcactggaggtagcacaaagtacgcagactccgtgaagggccggttcaccatctccagagacaattccaagaacacgctgtatctgcagatgaacagcctgagagccgaggacacggccgtatattactgtgcgcgtggttggccatctccagttactttcgactactggggccaaggaaccctggtcaccgtctcgagtggtggaggcggttcaggcggaggtggttctggcggtggcggatcggaaatcgtgttaacgcagtctccaggcaccctgtctttgtctccaggggaaagagccaccctctcttgcagggccagtcagagtgttagcagcagctacttagcctggtaccagcagaaacctggccaggctcccaggctcctcatctatggagcatccagcagggccactggcatcccagacaggttcagtggcagtggatccgggacagacttcactctcaccatcagcagactggagcctgaagattttgcagtgtattactgtcagcagtacaaatctcatccaatcacgttcggccaggggaccaaagtggaaatcaaacgt

SEQ ID NO: 84 - protein, 243 aa, synthetic construct
EVQLLESGGGLVQPGGSLRLSCAASGFTFSSYAMSWVRQAPGKGLEWVSAISGSGGSTYYADSVKGRFTISRDNSKNTLYLQMNSLRAEDTAVYYCARGWPSPVTFDYWGQGTLVTVSSGGGGSGGGGSGGGGSEIVLTQSPGTLSLSPGERATLSCRASQSVSRRYLAWYQQKPGQAPRLLIYGGSRRATGIPDRFSGSGSGTDFTLTISRLEPEDFAVYYCQQYKSHPITFGQGTKVEIKR

SEQ ID NO: 85 - DNA, 729 bp, synthetic construct
  source 1..729: mol_type = other DNA
gaggtgcaattgctggagtctgggggaggcttggtacagcctggggggtccctgagactctcctgtgcagcctccggattcacctttagcagttatgccatgagctgggtccgccaggctccagggaaggggctggagtgggtctcagctattagtggtagtggtggtagcacatactacgcagactccgtgaagggccggttcaccatctccagagacaattccaagaacacgctgtatctgcagatgaacagcctgagagccgaggacacggccgtatattactgtgcgcgtggttggccatctccagttactttcgactactggggccaaggaaccctggtcaccgtctcgagtggtggaggcggttcaggcggaggtggttctggcggtggcggatcggaaatcgtgttaacgcagtctccaggcaccctgtctttgtctccaggggaaagagccaccctctcttgcagggccagtcagagcgtcagtaggcgatacttagcctggtaccagcagaaacctggccaggctcccaggctcctcatctacggaggttcgcggagggccactggcatcccagacaggttcagtggcagtggatccgggacagacttcactctcaccatcagcagactggagcctgaagattttgcagtgtattactgtcagcagtacaaatctcatccaatcacgttcggccaggggaccaaagtggaaatcaaacgt

SEQ ID NO: 86 - protein, 243 aa, synthetic construct
EVQLLESGGGLVQPGGSLRLSCAASGFTFSRKALSWVRQAPGKGLEWVSTINGRGGRTYYADSVKGRFTISRDNSKNTLYLQMNSLRAEDTAVYYCARGWPSPVTFDYWGQGTLVTVSSGGGGSGGGGSGGGGSEIVLTQSPGTLSLSPGERATLSCRASQSVSSSYLAWYQQKPGQAPRLLIYGASSRATGIPDRFSGSGSGTDFTLTISRLEPEDFAVYYCQQYKSHPITFGQGTKVEIKR

SEQ ID NO: 87 - DNA, 729 bp, synthetic construct
  source 1..729: mol_type = other DNA
gaggtgcaattgctggagtctgggggaggcttggtacagcctggggggtccctgagactctcctgtgcagcctccggattcacctttagcagaaaggccctaagctgggtccgccaggctccagggaaggggctggagtgggtctcaactattaatggtagaggtggtcgcacatactacgcagactccgtgaagggccggttcaccatctccagagacaattccaagaacacgctgtatctgcagatgaacagcctgagagccgaggacacggccgtatattactgtgcgcgtggttggccatctccagttactttcgactactggggccaaggaaccctggtcaccgtctcgagtggtggaggcggttcaggcggaggtggttctggcggtggcggatcggaaatcgtgttaacgcagtctccaggcaccctgtctttgtctccaggggaaagagccaccctctcttgcagggccagtcagagtgttagcagcagctacttagcctggtaccagcagaaacctggccaggctcccaggctcctcatctatggagcatccagcagggccactggcatcccagacaggttcagtggcagtggatccgggacagacttcactctcaccatcagcagactggagcctgaagattttgcagtgtattactgtcagcagtacaaatctcatccaatcacgttcggccaggggaccaaagtggaaatcaaacgt

SEQ ID NO: 88 - protein, 467 aa, synthetic construct
EVQLLESGGGLVQPGGSLRLSCAASGFTFRRYAISWVRQAPGKGLEWVSAISGTGGSTKYADSVKGRFTISRDNSKNTLYLQMNSLRAEDTAVYYCARGWPSPVTFDYWGQGTLVTVSSGGGGSGGGGSGGGGSEIVLTQSPGTLSLSPGERATLSCRASQSVSSSYLAWYQQKPGQAPRLLIYGASSRATGIPDRFSGSGSGTDFTLTISRLEPEDFAVYYCQQYKSHPITFGQGTKVEIKRTTTPAPRPPTPAPTIASQPLSLRPEACRPAAGGAVHTRGLDFACDIYIWAPLAGTCGVLLLSLVITLYCKRGRKKLLYIFKQPFMRPVQTTQEEDGCSCRFPEEEEGGCELRVKFSRSADAPAYQQGQNQLYNELNLGRREEYDVLDKRRGRDPEMGGKPQRRKNPQEGLYNELQKDKMAEAYSEIGMKGERRRGKGHDGLYQGLSTATKDTYDALHMQALPPR

SEQ ID NO: 89 - protein, 467 aa, synthetic construct
EVQLLESGGGLVQPGGSLRLSCAASGFTFSSYAMSWVRQAPGKGLEWVSAISGSGGSTYYADSVKGRFTISRDNSKNTLYLQMNSLRAEDTAVYYCARGWPSPVTFDYWGQGTLVTVSSGGGGSGGGGSGGGGSEIVLTQSPGTLSLSPGERATLSCRASQSVSRRYLAWYQQKPGQAPRLLIYGGSRRATGIPDRFSGSGSGTDFTLTISRLEPEDFAVYYCQQYKSHPITFGQGTKVEIKRTTTPAPRPPTPAPTIASQPLSLRPEACRPAAGGAVHTRGLDFACDIYIWAPLAGTCGVLLLSLVITLYCKRGRKKLLYIFKQPFMRPVQTTQEEDGCSCRFPEEEEGGCELRVKFSRSADAPAYQQGQNQLYNELNLGRREEYDVLDKRRGRDPEMGGKPQRRKNPQEGLYNELQKDKMAEAYSEIGMKGERRRGKGHDGLYQGLSTATKDTYDALHMQALPPR

SEQ ID NO: 90 - protein, 467 aa, synthetic construct
EVQLLESGGGLVQPGGSLRLSCAASGFTFSRKALSWVRQAPGKGLEWVSTINGRGGRTYYADSVKGRFTISRDNSKNTLYLQMNSLRAEDTAVYYCARGWPSPVTFDYWGQGTLVTVSSGGGGSGGGGSGGGGSEIVLTQSPGTLSLSPGERATLSCRASQSVSSSYLAWYQQKPGQAPRLLIYGASSRATGIPDRFSGSGSGTDFTLTISRLEPEDFAVYYCQQYKSHPITFGQGTKVEIKRTTTPAPRPPTPAPTIASQPLSLRPEACRPAAGGAVHTRGLDFACDIYIWAPLAGTCGVLLLSLVITLYCKRGRKKLLYIFKQPFMRPVQTTQEEDGCSCRFPEEEEGGCELRVKFSRSADAPAYQQGQNQLYNELNLGRREEYDVLDKRRGRDPEMGGKPQRRKNPQEGLYNELQKDKMAEAYSEIGMKGERRRGKGHDGLYQGLSTATKDTYDALHMQALPPR

SEQ ID NO: 91 - protein, 227 aa, synthetic construct
DKTHTCPPCPAPELLGGPSVFLFPPKPKDTLMISRTPEVTCVVVDVSHEDPEVKFNWYVDGVEVHNAKTKPREEQYNSTYRVVSVLTVLHQDWLNGKEYKCKVSNKALPAPIEKTISKAKGQPREPQVYTLPPSRDELTKNQVSLTCLVKGFYPSDIAVEWESNGQPENNYKTTPPVLDSDGSFFLYSKLTVDKSRWQQGNVFSCSVMHEALHNHYTQKSLSLSPGK